European Patent Specification EP 3 578 646 B1, published July 15, 2026. Title: RATIONALLY-DESIGNED SINGLE-CHAIN MEGANUCLEASES WITH NON-PALINDROMIC RECOGNITION SEQUENCES. Applicant: PRECISION BIOSCIENCES, Inc. The sequence listing filed with the application follows.

SEQUENCE LISTING (110 sequences)

SEQ ID NO: 1 - protein, 163 aa, Chlamydomonas reinhardtii
MNTKYNKEFLLYLAGFVDGDGSIIAQIKPNQSYKFKHQLSLTFQVTQKTQRRWFLDKLVDEIGVGYVRDRGSVSDYILSEIKPLHNFLTQLQPFLKLKQKQANLVLKIIWRLPSAKESPDKFLEVCTWVDQIAALNDSKTRKTTSETVRAVLDSLSEKKKSSP

SEQ ID NO: 2 - protein, 170 aa, Monomastix sp.
MTTKNTLQPTEAAYIAGFLDGDGSIYAKLIPRPDYKDIKYQVSLAISFIQRKDKFPYLQDIYDQLGKRGNLRKDRGDGIADYTIIGSTHLSIILPDLVPYLRIKKKQANRILHIINLYPQAQKNPSKFLDLVKIVDDVQNLNKRADELKSTNYDRLLEEFLKAGKIESSP

SEQ ID NO: 3 - protein, 218 aa, Chlamydomonas moewusii
MSNFILKPGEKLPQDKLEELKKINDAVKKTKNFSKYLIDLRKLFQIDEVQVTSESKLFLAGFLEGEASLNISTKKLATSKFGLVVDPEFNVTQHVNGVKVLYLALEVFKTGRIRHKSGSNATLVLTIDNRQSLEEKVIPFYEQYVVAFSSPEKVKRVANFKALLELFNNDAHQDLEQLVNKILPIWDQMRKQQGQSNEGFPNLEAAQDFARNYKKGIK

SEQ ID NO: 4 - protein, 194 aa, Desulfurococcus mobilis
MHNNENVSGISAYLLGLIIGDGGLYKLKYKGNRSEYRVVITQKSENLIKQHIAPLMQFLIDELNVKSKIQIVKGDTRYELRVSSKKLYYYFANMLERIRLFNMREQIAFIKGLYVAEGDKTLKRLRIWNKNKALLEIVSRWLNNLGVRNTIHLDDHRHGVYVLNISLRDRIKFVHTILSSHLNPLPPERAGGYT

SEQ ID NO: 5 - protein, 235 aa, Saccharomyces cerevisiae
MKNIKKNQVMNLGPNSKLLKEYKSQLIELNIEQFEAGIGLILGDAYIRSRDEGKTYCMQFEWKNKAYMDHVCLLYDQWVLSPPHKKERVNHLGNLVITWGAQTFKHQAFNKLANLFIVNNKKTIPNNLVENYLTPMSLAYWFMDDGGKWDYNKNSTNKSIVLNTQSFTFEEVEYLVKGLRNKFQLNCYVKINKNKPIIYIDSMSYLIFYNLIKPYLIPQMMYKLPNTISSETFLK

SEQ ID NO: 6 - protein, 254 aa, Emericella nidulans
MSDLTYAYLVGLFEGDGYFSITKKGKYLTYELGIELSIKDVQLIYKIKKILGIGIVSFRKINEIEMVALRIRDKNHLKSFILPIFEKYPMFSNKQYDYLRFRNALLSGIISLEDLPDYTRSDEPLNSIESIINTSYFSAWLVGFIEAEGCFSVYKLNKDDDYLIASFDIAQRDGDILISAIRKYLSFTTKVYLDKTNCSKLKVTSVRSVENIIKFLQNAPVKLLGNKKLQYLLWLKQLRKISRYSEKIKIPSNY

SEQ ID NO: 7 - DNA, 9 bp, Chlamydomonas reinhardtii
gaaactgtc

SEQ ID NO: 8 - DNA, 9 bp, Chlamydomonas reinhardtii
gacagtttc

SEQ ID NO: 9 - DNA, 9 bp, Chlamydomonas reinhardtii
caaaacgtc

SEQ ID NO: 10 - DNA, 9 bp, Chlamydomonas reinhardtii
gacgttttg

SEQ ID NO: 11 - DNA, 9 bp, Monomastix sp.
cagaacgtc

SEQ ID NO: 12 - DNA, 9 bp, Monomastix sp.
gacgttctg

SEQ ID NO: 13 - DNA, 9 bp, Monomastix sp.
ggaactgtc

SEQ ID NO: 14 - DNA, 9 bp, Monomastix sp.
gacagttcc

SEQ ID NO: 15 - DNA, 9 bp, Chlamydomonas moewusii
ataacggtc

SEQ ID NO: 16 - DNA, 9 bp, Chlamydomonas moewusii
gaccgttat

SEQ ID NO: 17 - DNA, 9 bp, Chlamydomonas moewusii
ttcgctacc

SEQ ID NO: 18 - DNA, 9 bp, Chlamydomonas moewusii
ggtagcgaa

SEQ ID NO: 19 - DNA, 5 bp, Saccharomyces cerevisiae
taggg

SEQ ID NO: 20 - DNA, 5 bp, Saccharomyces cerevisiae
cccta

SEQ ID NO: 21 - DNA, 9 bp, Saccharomyces cerevisiae
taatgggac

SEQ ID NO: 22 - DNA, 9 bp, Saccharomyces cerevisiae
gtcccatta

SEQ ID NO: 23 - DNA, 8 bp, Desulfurococcus mobilis
gccggaac

SEQ ID NO: 24 - DNA, 8 bp, Desulfurococcus mobilis
gttccggc

SEQ ID NO: 25 - DNA, 7 bp, Desulfurococcus mobilis
aacggcc

SEQ ID NO: 26 - DNA, 7 bp, Desulfurococcus mobilis
ggccgtt

SEQ ID NO: 27 - DNA, 8 bp, Emericella nidulans
tttacaga

SEQ ID NO: 28 - DNA, 8 bp, Emericella nidulans
tctgtaaa

SEQ ID NO: 29 - DNA, 9 bp, Emericella nidulans
ctgaggagg

SEQ ID NO: 30 - DNA, 9 bp, Emericella nidulans
cctcctcag

SEQ ID NO: 31 - protein, 163 aa, Artificial Sequence
  Description of Artificial Sequence: Synthetic polypeptide
MNTKYNKEFLLYLAGFVDGDGSIKAQIKPEQNRKFKHRLELTFQVTQKTQRRWFLDKLVDEIGVGYVYDRGSVSDYILSEIKPLHNFLTQLQPFLKLKQKQANLVLKIIWRLPSAKESPDKFLEVCTWVDQIAALNDSKTRKTTSETVRAVLDSLSEKKKSSP

SEQ ID NO: 32 - DNA, 22 bp, Artificial Sequence
  Description of Artificial Sequence: Synthetic oligonucleotide
aggcatctcattagagatgcct

SEQ ID NO: 33 - DNA, 22 bp, Artificial Sequence
  Description of Artificial Sequence: Synthetic oligonucleotide
aggcatctctaatgagatgcct

SEQ ID NO: 34 - DNA, 22 bp, Chlamydomonas reinhardtii
gaaactgtctcacgacgttttg

SEQ ID NO: 35 - DNA, 22 bp, Chlamydomonas reinhardtii
caaaacgtcgtgagacagtttc

SEQ ID NO: 36 - protein, 163 aa, Artificial Sequence
  Description of Artificial Sequence: Synthetic polypeptide
MNTKYNKEFLLYLAGFVDGDGSIIAQIDPRQCRKFKHELRLRFQVTQKTQRRWFLDKLVDEIGVGYVRDRGSVSDYILSEIKPLHNFLTQLQPFLKLKQKQANLVLKIIWRLPSAKESPDKFLEVCTWVDQIAALNDSKTRKTTSETVRAVLDSLSEKKKSSP

SEQ ID NO: 37 - protein, 163 aa, Artificial Sequence
  Description of Artificial Sequence: Synthetic polypeptide
MNTKYNKEFLLYLAGFVDGDGSIIAQIKPEQSYKFKHRLRLEFQVTQKTQRRWFLDKLVDEIGVGYVRDRGSVSDYILSEIKPLHNFLTQLQPFLKLKQKQANLVLKIIWRLPSAKESPDKFLEVCTWVDQIAALNDSKTRKTTSETVRAVLDSLSEKKKSSP

SEQ ID NO: 38 - DNA, 9 bp, Artificial Sequence
  Description of Artificial Sequence: Synthetic oligonucleotide
tgcggtgtc

SEQ ID NO: 39 - DNA, 9 bp, Artificial Sequence
  Description of Artificial Sequence: Synthetic oligonucleotide
gacaccgca

SEQ ID NO: 40 - DNA, 22 bp, Artificial Sequence
  Description of Artificial Sequence: Synthetic oligonucleotide
  modified_base (10)..(13): a, c, t, g, u, unknown or other
tgcggtgtcnnnngacaccgca

SEQ ID NO: 41 - DNA, 22 bp, Artificial Sequence
  Description of Artificial Sequence: Synthetic oligonucleotide
  modified_base (10)..(13): a, c, t, g, u, unknown or other
tgcggtgtcnnnngacaccgca

SEQ ID NO: 42 - DNA, 9 bp, Artificial Sequence
  Description of Artificial Sequence: Synthetic oligonucleotide
caggctgtc

SEQ ID NO: 43 - DNA, 9 bp, Artificial Sequence
  Description of Artificial Sequence: Synthetic oligonucleotide
gacagcctg

SEQ ID NO: 44 - DNA, 22 bp, Artificial Sequence
  Description of Artificial Sequence: Synthetic oligonucleotide
  modified_base (10)..(13): a, c, t, g, u, unknown or other
caggctgtcnnnngacagcctg

SEQ ID NO: 45 - DNA, 22 bp, Artificial Sequence
  Description of Artificial Sequence: Synthetic oligonucleotide
  modified_base (10)..(13): a, c, t, g, u, unknown or other
caggctgtcnnnngacagcctg

SEQ ID NO: 46 - DNA, 22 bp, Artificial Sequence
  Description of Artificial Sequence: Synthetic oligonucleotide
tgcggtgtcattagacagcctg

SEQ ID NO: 47 - DNA, 22 bp, Artificial Sequence
  Description of Artificial Sequence: Synthetic oligonucleotide
caggctgtctaatgacaccgca

SEQ ID NO: 48 - protein, 260 aa, Artificial Sequence
  Description of Artificial Sequence: Synthetic polypeptide
MNTKYNKEFLLYLAGFVDGDGSIIAQIDPRQCRKFKHELRLRFQVTQKTQRRWFLDKLVDEIGVGYVRDRGSVSDYILSEIKPLHNFLTQLQPMLERIRLFNMREFLLYLAGFVDGDGSIIAQIKPEQSYKFKHRLRLEFQVTQKTQRRWFLDKLVDEIGVGYVRDRGSVSDYILSEIKPLHNFLTQLQPFLKLKQKQANLVLKIIWRLPSAKESPDKFLEVCTWVDQIAALNDSKTRKTTSETVRAVLDSLSEKKKSSP

SEQ ID NO: 49 - protein, 260 aa, Artificial Sequence
  Description of Artificial Sequence: Synthetic polypeptide
MNTKYNKEFLLYLAGFVDGDGSIIAQIKPEQSYKFKHRLRLEFQVTQKTQRRWFLDKLVDEIGVGYVRDRGSVSDYILSEIKPLHNFLTQLQPMLERIRLFNMREFLLYLAGFVDGDGSIIAQIDPRQCRKFKHELRLRFQVTQKTQRRWFLDKLVDEIGVGYVRDRGSVSDYILSEIKPLHNFLTQLQPFLKLKQKQANLVLKIIWRLPSAKESPDKFLEVCTWVDQIAALNDSKTRKTTSETVRAVLDSLSEKKKSSP

SEQ ID NO: 50 - protein, 334 aa, Artificial Sequence
  Description of Artificial Sequence: Synthetic polypeptide
MNTKYNKEFLLYLAGFVDGDGSIIAQIDPRQCRKFKHELRLRFQVTQKTQRRWFLDKLVDEIGVGYVRDRGSVSDYILSEIKPLHNFLTQLQPFLKLKQKQANLVLKIIWRLPSAKESPDKFLEVCTWVDQIAALNDSKTRKTTSETVRAVGSSGSSGSSGSSGSSGSSGSSGSSGSSGFLLYLAGFVDGDGSIIAQIKPEQSYKFKHRLRLEFQVTQKTQRRWFLDKLVDEIGVGYVRDRGSVSDYILSEIKPLHNFLTQLQPFLKLKQKQANLVLKIIWRLPSAKESPDKFLEVCTWVDQIAALNDSKTRKTTSETVRAVLDSLSEKKKSSP

SEQ ID NO: 51 - protein, 350 aa, Artificial Sequence
  Description of Artificial Sequence: Synthetic polypeptide
MNTKYNKEFLLYLAGFVDGDGSIIAQIDPRQCRKFKHELRLRFQVTQKTQRRWFLDKLVDEIGVGYVRDRGSVSDYILSEIKPLHNFLTQLQPFLKLKQKQANLVLKIIWRLPSAKESPDKFLEVCTWVDQIAALNDSKTRKTTSETVRAVLDSLPGSVGGLSPSQASSAASSASSSPGSGISEALRAGATKSKEFLLYLAGFVDGDGSIIAQIKPEQSYKFKHRLRLEFQVTQKTQRRWFLDKLVDEIGVGYVRDRGSVSDYILSEIKPLHNFLTQLQPFLKLKQKQANLVLKIIWRLPSAKESPDKFLEVCTWVDQIAALNDSKTRKTTSETVRAVLDSLSEKKKSSP

SEQ ID NO: 52 - protein, 373 aa, Artificial Sequence
  Description of Artificial Sequence: Synthetic polypeptide
MTTKNTLQPTEAAYIAGFLDGDGSIYAKLIPRPDYKDIKYQVSLAISFIQRKDKFPYLQDIYDQLGKRGNLRKDRGDGIADYTIIGSTHLSIILPDLVPYLRIKKKQANRILHIINLYPQAQKNPSKFLDLVKIVDDVQNLNKRADELKSTNYDRLLEEFLKAGKIGGASPSQASSAASSASSAASSPGSGPSEALRAASSFASKPGSTLQPTEAAYIAGFLDGDGSIYAKLIPRPDYKDIKYQVSLAISFIQRKDKFPYLQDIYDQLGKRGNLRKDRGDGIADYTIIGSTHLSIILPDLVPYLRIKKKQANRILHIINLYPQAQKNPSKFLDLVKIVDDVQNLNKRADELKSTNYDRLLEEFLKAGKIESSP

SEQ ID NO: 53 - DNA, 22 bp, Monomastix sp.
ggaactgtctcacgacgttctg

SEQ ID NO: 54 - DNA, 22 bp, Monomastix sp.
cagaacgtcgtgagacagttcc

SEQ ID NO: 55 - protein, 9 aa, Artificial Sequence
  Description of Artificial Sequence: Synthetic peptide
LAGLIDADG

SEQ ID NO: 56 - DNA, 22 bp, Artificial Sequence
  Description of Artificial Sequence: Synthetic oligonucleotide
  modified_base (10)..(13): a, c, t, g, u, unknown or other
tgcggtgtcnnnngacagcctg

SEQ ID NO: 57 - DNA, 22 bp, Artificial Sequence
  Description of Artificial Sequence: Synthetic oligonucleotide
  modified_base (10)..(13): a, c, t, g, u, unknown or other
caggctgtcnnnngacaccgca

SEQ ID NO: 58 - protein, 4 aa, Artificial Sequence
  Description of Artificial Sequence: Synthetic peptide
SGGS

SEQ ID NO: 59 - protein, 22 aa, Artificial Sequence
  Description of Artificial Sequence: Synthetic peptide
GSSGSSGSSGSSGSSGSSGSSG

SEQ ID NO: 60 - protein, 25 aa, Artificial Sequence
  Description of Artificial Sequence: Synthetic peptide
GSSGSSGSSGSSGSSGSSGSSGSSG

SEQ ID NO: 61 - protein, 28 aa, Artificial Sequence
  Description of Artificial Sequence: Synthetic peptide
GSSGSSGSSGSSGSSGSSGSSGSSGSSG

SEQ ID NO: 62 - protein, 31 aa, Artificial Sequence
  Description of Artificial Sequence: Synthetic polypeptide
GSSGSSGSSGSSGSSGSSGSSGSSGSSGSSG

SEQ ID NO: 63 - protein, 34 aa, Artificial Sequence
  Description of Artificial Sequence: Synthetic polypeptide
GSSGSSGSSGSSGSSGSSGSSGSSGSSGSSGSSG

SEQ ID NO: 64 - protein, 29 aa, Artificial Sequence
  Description of Artificial Sequence: Synthetic peptide
GSSGSSGSSGSSGSSGSSGSSGSSGSSGG

SEQ ID NO: 65 - protein, 30 aa, Artificial Sequence
  Description of Artificial Sequence: Synthetic polypeptide
GSSGSSGSSGSSGSSGSSGSSGSSGSSGSG

SEQ ID NO: 66 - protein, 8 aa, Artificial Sequence
  Description of Artificial Sequence: Synthetic peptide
VLDSPGSV

SEQ ID NO: 67 - protein, 12 aa, Artificial Sequence
  Description of Artificial Sequence: Synthetic peptide
SQASSAASSASS

SEQ ID NO: 68 - protein, 6 aa, Artificial Sequence
  Description of Artificial Sequence: Synthetic peptide
LSPSQA

SEQ ID NO: 69 - protein, 9 aa, Artificial Sequence
  Description of Artificial Sequence: Synthetic peptide
ASSSPGSGI

SEQ ID NO: 70 - protein, 4 aa, Artificial Sequence
  Description of Artificial Sequence: Synthetic peptide
ASSS

SEQ ID NO: 71 - protein, 5 aa, Artificial Sequence
  Description of Artificial Sequence: Synthetic peptide
PGSGI

SEQ ID NO: 72 - protein, 6 aa, Artificial Sequence
  Description of Artificial Sequence: Synthetic peptide
ISEALR

SEQ ID NO: 73 - protein, 6 aa, Artificial Sequence
  Description of Artificial Sequence: Synthetic peptide
SEALRA

SEQ ID NO: 74 - protein, 4 aa, Artificial Sequence
  Description of Artificial Sequence: Synthetic peptide
ASSA

SEQ ID NO: 75 - protein, 6 aa, Artificial Sequence
  Description of Artificial Sequence: Synthetic peptide
ALRAGA

SEQ ID NO: 76 - protein, 6 aa, Artificial Sequence
  Description of Artificial Sequence: Synthetic peptide
TKSKEF

SEQ ID NO: 77 - protein, 40 aa, Artificial Sequence
  Description of Artificial Sequence: Synthetic polypeptide
SLPGSVGGLSPSQASSAASSASSSPGSGISEALRAGATKS

SEQ ID NO: 78 - protein, 41 aa, Artificial Sequence
  Description of Artificial Sequence: Synthetic polypeptide
SLPGSVGGLSPSQASSAASSASSSPGSGISEALRAGGATKS

SEQ ID NO: 79 - protein, 42 aa, Artificial Sequence
  Description of Artificial Sequence: Synthetic polypeptide
SLPGSVGGLSPSQASSAASSASSSPGSGISEALRAAGGATKS

SEQ ID NO: 80 - protein, 43 aa, Artificial Sequence
  Description of Artificial Sequence: Synthetic polypeptide
SLPGSVGGLSPSQASSAASSASSSPGSGISEALRAASGGATKS

SEQ ID NO: 81 - protein, 44 aa, Artificial Sequence
  Description of Artificial Sequence: Synthetic polypeptide
SLPGSVGGLSPSQASSAASSASSSPGSGISEALRAASSGGATKS

SEQ ID NO: 82 - protein, 45 aa, Artificial Sequence
  Description of Artificial Sequence: Synthetic polypeptide
SLPGSVGGLSPSQASSAASSASSSPGSGISEALRAASSAGGATKS

SEQ ID NO: 83 - protein, 41 aa, Artificial Sequence
  Description of Artificial Sequence: Synthetic polypeptide
SLPGSVGGLSPSQASSAASSASSSPGSGISEALRAGATKEF

SEQ ID NO: 84 - protein, 41 aa, Artificial Sequence
  Description of Artificial Sequence: Synthetic polypeptide
SLPGSVGGISPSQASSAASSASSSPGSGTSEAPRAGATKEF

SEQ ID NO: 85 - protein, 41 aa, Artificial Sequence
  Description of Artificial Sequence: Synthetic polypeptide
SLPGSVGGLSPSQASSAASSASSSPGSGTSEATRAGATKEF

SEQ ID NO: 86 - protein, 41 aa, Artificial Sequence
  Description of Artificial Sequence: Synthetic polypeptide
SLPGSLGGLSPSQASSAASSASSSPGSGPSEALRAGATKEF

SEQ ID NO: 87 - protein, 41 aa, Artificial Sequence
  Description of Artificial Sequence: Synthetic polypeptide
SLPGSVGGVSPSQASSAASSASSSPGSGVSEASRAGATKEF

SEQ ID NO: 88 - protein, 41 aa, Artificial Sequence
  Description of Artificial Sequence: Synthetic polypeptide
SLPGSVGGLSPSQASSAASSASSSPGSGLSEALRAGATKEF

SEQ ID NO: 89 - protein, 41 aa, Artificial Sequence
  Description of Artificial Sequence: Synthetic polypeptide
SLPGSLGGISPSQASSAASSASSSPGSGSSEASRAGATKEF

SEQ ID NO: 90 - protein, 40 aa, Artificial Sequence
  Description of Artificial Sequence: Synthetic polypeptide
SPGSVGGVSPSQASSAASSASSSPGSGISEATRAGATKEF

SEQ ID NO: 91 - protein, 37 aa, Artificial Sequence
  Description of Artificial Sequence: Synthetic polypeptide
SLPGSLGGVSPSQASSAASSPGSGTSEAPRAGATKEF

SEQ ID NO: 92 - protein, 37 aa, Artificial Sequence
  Description of Artificial Sequence: Synthetic polypeptide
SLPGSVGGLSPSQASSAASSPGSGISEAIRAGATKEF

SEQ ID NO: 93 - protein, 44 aa, Artificial Sequence
  Description of Artificial Sequence: Synthetic polypeptide
SLPGSLGGVSPSQASSAASSASSAASSPGSGASEASRAGATKEF

SEQ ID NO: 94 - protein, 6 aa, Monomastix sp.
LQPTEA

SEQ ID NO: 95 - protein, 39 aa, Artificial Sequence
  Description of Artificial Sequence: Synthetic polypeptide
PGSVGGLSPSQASSAASSASSSPGSGISEALRAGATKSA

SEQ ID NO: 96 - protein, 39 aa, Artificial Sequence
  Description of Artificial Sequence: Synthetic polypeptide
PGSVGGLSPSQASSAASSASSSPGSGISEALRAGATKSG

SEQ ID NO: 97 - protein, 43 aa, Artificial Sequence
  Description of Artificial Sequence: Synthetic polypeptide
GGASPSQASSAASSASSAASSPGSGISEALRAASSLASKPGST

SEQ ID NO: 98 - protein, 39 aa, Artificial Sequence
  Description of Artificial Sequence: Synthetic polypeptide
GGASPSQASSAASSASSAASSPGSGISEALRAASSPGST

SEQ ID NO: 99 - protein, 43 aa, Artificial Sequence
  Description of Artificial Sequence: Synthetic polypeptide
GGASPSQASSAASSASSAASSPGSGPSEALRAASSFASKPGST

SEQ ID NO: 100 - protein, 4 aa, Artificial Sequence
  Description of Artificial Sequence: Synthetic peptide
LPGE

SEQ ID NO: 101 - protein, 13 aa, Artificial Sequence
  Description of Artificial Sequence: Synthetic peptide
GSSGSSGSSGSSG

SEQ ID NO: 102 - protein, 16 aa, Artificial Sequence
  Description of Artificial Sequence: Synthetic peptide
GSSGSSGSSGSSGSSG

SEQ ID NO: 103 - protein, 29 aa, Artificial Sequence
  Description of Artificial Sequence: Synthetic peptide
NSLPGSVGGLSPSQASSAASSASSSPGSG

SEQ ID NO: 104 - protein, 11 aa, Desulfurococcus mobilis
MLERIRLFNMR

SEQ ID NO: 105 - DNA, 22 bp, Artificial Sequence
  Description of Artificial Sequence: Synthetic oligonucleotide
tgcggtgtcattagacaccgca

SEQ ID NO: 106 - DNA, 22 bp, Artificial Sequence
  Description of Artificial Sequence: Synthetic oligonucleotide
tgcggtgtctaatgacaccgca

SEQ ID NO: 107 - DNA, 22 bp, Artificial Sequence
  Description of Artificial Sequence: Synthetic oligonucleotide
caggctgtcattagacagcctg

SEQ ID NO: 108 - DNA, 22 bp, Artificial Sequence
  Description of Artificial Sequence: Synthetic oligonucleotide
caggctgtcattagacagcctg

SEQ ID NO: 109 - protein, 46 aa, Artificial Sequence
  Description of Artificial Sequence: Synthetic polypeptide
VLDSLPGSVGGLSPSQASSAASSASSSPGSGISEALRAGATKSKEF

SEQ ID NO: 110 - protein, 6 aa, Artificial Sequence
  Description of Artificial Sequence: Synthetic 6xHis tag
HHHHHH